European Patent Application EP 4 442 828 A1, published October 9, 2024. Title: PROTEASE-CLEAVABLE MASKED ANTIBODIES. Applicant: Daiichi Sankyo Company, Limited. Application EP 22901261.2, filed November 29, 2022. The sequence listing filed with the application follows.

SEQUENCE LISTING (64 sequences)

SEQ ID NO: 1 - protein, 470 aa, synthetic construct
  REGION 1..470: note = Amino acid sequence of the full length of HT1-11 H chain
MKHLWFFLLLVAAPRWVLSQVQLVQSGAEVKKPGASVKVSCKASGYTFTTAGMQWVRQAPGQGLEWMGWINTHSGVPKYAEDFKGRVTISADTSTSTAYLQLSSLKSEDTAVYYCARSGFGSSYWYFDVWGQGTLVTVSSASTKGPSVFPLAPSSKSTSGGTAALGCLVKDYFPEPVTVSWNSGALTSGVHTFPAVLQSSGLYSLSSVVTVPSSSLGTQTYICNVNHKPSNTKVDKRVEPKSCDKTHTCPPCPAPELLGGPSVFLFPPKPKDTLMISRTPEVTCVVVDVSHEDPEVKFNWYVDGVEVHNAKTKPREEQYNSTYRVVSVLTVLHQDWLNGKEYKCKVSNKALPAPIEKTISKAKGQPREPQVYTLPPSREEMTKNQVSLTCLVKGFYPSDIAVEWESNGQPENNYKTTPPVLDSDGSFFLYSKLTVDKSRWQQGNVFSCSVMHEALHNHYTQKSLSLSPGK

SEQ ID NO: 2 - protein, 234 aa, synthetic construct
  REGION 1..234: note = Amino acid sequence of the full length of HT1-11 Lchain
MVLQTQVFISLLLWISGAYGDIQMTQSPSSLSASVGDRVTITCKASQDVSTAVAWYQQKPGKAPKLLIYSASYRYTGVPSRFSGSGSGTDFTLTISSLQPEDFAVYYCQQHYITPLTFGQGTKLEIKRTVAAPSVFIFPPSDEQLKSGTASVVCLLNNFYPREAKVQWKVDNALQSGNSQESVTEQDSKDSTYSLSSTLTLSKADYEKHKVYACEVTHQGLSSPVTKSFNRGEC

SEQ ID NO: 3 - protein, 331 aa, synthetic construct
  REGION 1..331: note = Amino acid sequence of the full length of MHT1001
MKYLLPTAAAGLLLLAAQPAMAAMGYLALKHPWPGLAENSGSGGGGSVLVPMAMMASGGSDVNSQVQLVQSGAEVKKPGASVKVSCKASGYTFTTAGMQWVRQAPGQGLEWMGWINTHSGVPKYAEDFKGRVTISADTSTSTAYLQLSSLKSEDTAVYYCARSGFGSSYWYFDVWGQGTLVTVSSGGGGSGGGGSGGGGSDIQMTQSPSSLSASVGDRVTITCKASQDVSTAVAWYQQKPGKAPKLLIYSASYRYTGVPSRFSGSGSGTDFTLTISSLQPEDFAVYYCQQHYITPLTFGQGTKLEIKRGAPSGDYKDDDDKGAAAHHHHHH

SEQ ID NO: 4 - protein, 331 aa, synthetic construct
  REGION 1..331: note = Amino acid sequence of the full length of MHT1002
MKYLLPTAAAGLLLLAAQPAMAAMGYLALKHPWPGLAENSGSGGGGSVLVPMAMMASGGSDVNSDIQMTQSPSSLSASVGDRVTITCKASQDVSTAVAWYQQKPGKAPKLLIYSASYRYTGVPSRFSGSGSGTDFTLTISSLQPEDFAVYYCQQHYITPLTFGQGTKLEIKRGGGGSGGGGSGGGGSQVQLVQSGAEVKKPGASVKVSCKASGYTFTTAGMQWVRQAPGQGLEWMGWINTHSGVPKYAEDFKGRVTISADTSTSTAYLQLSSLKSEDTAVYYCARSGFGSSYWYFDVWGQGTLVTVSSGAPSGDYKDDDDKGAAAHHHHHH

SEQ ID NO: 5 - protein, 294 aa, synthetic construct
  REGION 1..294: note = Amino acid sequence of the full length of HT1-11-scFv-HL
MKYLLPTAAAGLLLLAAQPAMAADVNSQVQLVQSGAEVKKPGASVKVSCKASGYTFTTAGMQWVRQAPGQGLEWMGWINTHSGVPKYAEDFKGRVTISADTSTSTAYLQLSSLKSEDTAVYYCARSGFGSSYWYFDVWGQGTLVTVSSGGGGSGGGGSGGGGSDIQMTQSPSSLSASVGDRVTITCKASQDVSTAVAWYQQKPGKAPKLLIYSASYRYTGVPSRFSGSGSGTDFTLTISSLQPEDFAVYYCQQHYITPLTFGQGTKLEIKRGAPSGDYKDDDDKGAAAHHHHHH

SEQ ID NO: 6 - protein, 294 aa, synthetic construct
  REGION 1..294: note = Amino acid sequence of the full length of HT1-11-scFv-LH
MKYLLPTAAAGLLLLAAQPAMAADVNSDIQMTQSPSSLSASVGDRVTITCKASQDVSTAVAWYQQKPGKAPKLLIYSASYRYTGVPSRFSGSGSGTDFTLTISSLQPEDFAVYYCQQHYITPLTFGQGTKLEIKRGGGGSGGGGSGGGGSQVQLVQSGAEVKKPGASVKVSCKASGYTFTTAGMQWVRQAPGQGLEWMGWINTHSGVPKYAEDFKGRVTISADTSTSTAYLQLSSLKSEDTAVYYCARSGFGSSYWYFDVWGQGTLVTVSSGAPSGDYKDDDDKGAAAHHHHHH

SEQ ID NO: 7 - protein, 506 aa, synthetic construct
  REGION 1..506: note = Amino acid sequence of the full length of MHT1007 H chain
MKHLWFFLLLVAAPRWVLSGYLALKHPWPGLAENSGSGGGGSVLVPMAMMASGGSQVQLVQSGAEVKKPGASVKVSCKASGYTFTTAGMQWVRQAPGQGLEWMGWINTHSGVPKYAEDFKGRVTISADTSTSTAYLQLSSLKSEDTAVYYCARSGFGSSYWYFDVWGQGTLVTVSSASTKGPSVFPLAPSSKSTSGGTAALGCLVKDYFPEPVTVSWNSGALTSGVHTFPAVLQSSGLYSLSSVVTVPSSSLGTQTYICNVNHKPSNTKVDKRVEPKSCDKTHTCPPCPAPELLGGPSVFLFPPKPKDTLMISRTPEVTCVVVDVSHEDPEVKFNWYVDGVEVHNAKTKPREEQYNSTYRVVSVLTVLHQDWLNGKEYKCKVSNKALPAPIEKTISKAKGQPREPQVYTLPPSREEMTKNQVSLTCLVKGFYPSDIAVEWESNGQPENNYKTTPPVLDSDGSFFLYSKLTVDKSRWQQGNVFSCSVMHEALHNHYTQKSLSLSPGK

SEQ ID NO: 8 - protein, 506 aa, synthetic construct
  REGION 1..506: note = Amino acid sequence of the full length of MHT1008 H chain
MKHLWFFLLLVAAPRWVLSGYLALKHPWPGLAENSGSGGGGSGGGGSGGGGSGGSQVQLVQSGAEVKKPGASVKVSCKASGYTFTTAGMQWVRQAPGQGLEWMGWINTHSGVPKYAEDFKGRVTISADTSTSTAYLQLSSLKSEDTAVYYCARSGFGSSYWYFDVWGQGTLVTVSSASTKGPSVFPLAPSSKSTSGGTAALGCLVKDYFPEPVTVSWNSGALTSGVHTFPAVLQSSGLYSLSSVVTVPSSSLGTQTYICNVNHKPSNTKVDKRVEPKSCDKTHTCPPCPAPELLGGPSVFLFPPKPKDTLMISRTPEVTCVVVDVSHEDPEVKFNWYVDGVEVHNAKTKPREEQYNSTYRVVSVLTVLHQDWLNGKEYKCKVSNKALPAPIEKTISKAKGQPREPQVYTLPPSREEMTKNQVSLTCLVKGFYPSDIAVEWESNGQPENNYKTTPPVLDSDGSFFLYSKLTVDKSRWQQGNVFSCSVMHEALHNHYTQKSLSLSPGK

SEQ ID NO: 9 - protein, 506 aa, synthetic construct
  REGION 1..506: note = Amino acid sequence of the full length of MHT1009 H chain
MKHLWFFLLLVAAPRWVLSGYLALKHPWPGLAENSGSGGSGGSGRSANAILEGGSQVQLVQSGAEVKKPGASVKVSCKASGYTFTTAGMQWVRQAPGQGLEWMGWINTHSGVPKYAEDFKGRVTISADTSTSTAYLQLSSLKSEDTAVYYCARSGFGSSYWYFDVWGQGTLVTVSSASTKGPSVFPLAPSSKSTSGGTAALGCLVKDYFPEPVTVSWNSGALTSGVHTFPAVLQSSGLYSLSSVVTVPSSSLGTQTYICNVNHKPSNTKVDKRVEPKSCDKTHTCPPCPAPELLGGPSVFLFPPKPKDTLMISRTPEVTCVVVDVSHEDPEVKFNWYVDGVEVHNAKTKPREEQYNSTYRVVSVLTVLHQDWLNGKEYKCKVSNKALPAPIEKTISKAKGQPREPQVYTLPPSREEMTKNQVSLTCLVKGFYPSDIAVEWESNGQPENNYKTTPPVLDSDGSFFLYSKLTVDKSRWQQGNVFSCSVMHEALHNHYTQKSLSLSPGK

SEQ ID NO: 10 - protein, 506 aa, synthetic construct
  REGION 1..506: note = Amino acid sequence of the full length of MHT3002 H chain
MKHLWFFLLLVAAPRWVLSGYLALKHPWPGLAEGSGGGGSGGGGSGPLFAARGGSQVQLVQSGAEVKKPGASVKVSCKASGYTFTTAGMQWVRQAPGQGLEWMGWINTHSGVPKYAEDFKGRVTISADTSTSTAYLQLSSLKSEDTAVYYCARSGFGSSYWYFDVWGQGTLVTVSSASTKGPSVFPLAPSSKSTSGGTAALGCLVKDYFPEPVTVSWNSGALTSGVHTFPAVLQSSGLYSLSSVVTVPSSSLGTQTYICNVNHKPSNTKVDKRVEPKSCDKTHTCPPCPAPELLGGPSVFLFPPKPKDTLMISRTPEVTCVVVDVSHEDPEVKFNWYVDGVEVHNAKTKPREEQYNSTYRVVSVLTVLHQDWLNGKEYKCKVSNKALPAPIEKTISKAKGQPREPQVYTLPPSREEMTKNQVSLTCLVKGFYPSDIAVEWESNGQPENNYKTTPPVLDSDGSFFLYSKLTVDKSRWQQGNVFSCSVMHEALHNHYTQKSLSLSPGK

SEQ ID NO: 11 - protein, 713 aa, synthetic construct
  REGION 1..713: note = Amino acid sequence of the full length of human CAPN1
SEEIITPVYCTGVSAQVQKQRARELGLGRHENAIKYLGQDYEQLRVRCLQSGTLFRDEAFPPVPQSLGYKDLGPNSSKTYGIKWKRPTELLSNPQFIVDGATRTDICQGALGDCWLLAAIASLTLNDTLLHRVVPHGQSFQNGYAGIFHFQLWQFGEWVDVVVDDLLPIKDGKLVFVHSAEGNEFWSALLEKAYAKVNGSYEALSGGSTSEGFEDFTGGVTEWYELRKAPSDLYQIILKALERGSLLGCSIDISSVLDMEAITFKKLVKGHAYSVTGAKQVNYRGQVVSLIRMRNPWGEVEWTGAWSDSSSEWNNVDPYERDQLRVKMEDGEFWMSFRDFMREFTRLEICNLTPDALKSRTIRKWNTTLYEGTWRRGSTAGGCRNYPATFWVNPQFKIRLDETDDPDDYGDRESGCSFVLALMQKHRRRERRFGRDMETIGFAVYEVPPELVGQPAVHLKRDFFLANASRARSEQFINLREVSTRFRLPPGEYVVVPSTFEPNKEGDFVLRFFSEKSAGTVELDDQIQANLPDEQVLSEEEIDENFKALFRQLAGEDMEISVKELRTILNRIISKHKDLRTKGFSLESCRSMVNLMDRDGNGKLGLVEFNILWNRIRNYLSIFRKFDLDKSGSMSAYEMRMAIESAGFKLNKKLYELIITRYSEPDLAVDFDNFVCCLVRLETMFRFFKTLDTDLDGVVTFDLFKWLQLTMFA

SEQ ID NO: 12 - protein, 6 aa, synthetic construct
  REGION 1..6: note = Amino acid sequence of a new CAPN substrate
PLFAAP

SEQ ID NO: 13 - protein, 506 aa, synthetic construct
  REGION 1..506: note = Amino acid sequence of the full length of MHT3201 H chain
MKHLWFFLLLVAAPRWVLSGYLALKHPWPGLAEGSGGGGSGGGGSGPLFAAPGGSQVQLVQSGAEVKKPGASVKVSCKASGYTFTTAGMQWVRQAPGQGLEWMGWINTHSGVPKYAEDFKGRVTISADTSTSTAYLQLSSLKSEDTAVYYCARSGFGSSYWYFDVWGQGTLVTVSSASTKGPSVFPLAPSSKSTSGGTAALGCLVKDYFPEPVTVSWNSGALTSGVHTFPAVLQSSGLYSLSSVVTVPSSSLGTQTYICNVNHKPSNTKVDKRVEPKSCDKTHTCPPCPAPELLGGPSVFLFPPKPKDTLMISRTPEVTCVVVDVSHEDPEVKFNWYVDGVEVHNAKTKPREEQYNSTYRVVSVLTVLHQDWLNGKEYKCKVSNKALPAPIEKTISKAKGQPREPQVYTLPPSREEMTKNQVSLTCLVKGFYPSDIAVEWESNGQPENNYKTTPPVLDSDGSFFLYSKLTVDKSRWQQGNVFSCSVMHEALHNHYTQKSLSLSPGK

SEQ ID NO: 14 - protein, 506 aa, synthetic construct
  REGION 1..506: note = Amino acid sequence of the full length of MHT3202 H chain
MKHLWFFLLLVAAPRWVLSGYLALKHPWPGLAEGSGGGGSGRSAGGPLFAAPGGSQVQLVQSGAEVKKPGASVKVSCKASGYTFTTAGMQWVRQAPGQGLEWMGWINTHSGVPKYAEDFKGRVTISADTSTSTAYLQLSSLKSEDTAVYYCARSGFGSSYWYFDVWGQGTLVTVSSASTKGPSVFPLAPSSKSTSGGTAALGCLVKDYFPEPVTVSWNSGALTSGVHTFPAVLQSSGLYSLSSVVTVPSSSLGTQTYICNVNHKPSNTKVDKRVEPKSCDKTHTCPPCPAPELLGGPSVFLFPPKPKDTLMISRTPEVTCVVVDVSHEDPEVKFNWYVDGVEVHNAKTKPREEQYNSTYRVVSVLTVLHQDWLNGKEYKCKVSNKALPAPIEKTISKAKGQPREPQVYTLPPSREEMTKNQVSLTCLVKGFYPSDIAVEWESNGQPENNYKTTPPVLDSDGSFFLYSKLTVDKSRWQQGNVFSCSVMHEALHNHYTQKSLSLSPGK

SEQ ID NO: 15 - protein, 506 aa, synthetic construct
  REGION 1..506: note = Amino acid sequence of the full length of MHT1713 H chain
MKHLWFFLLLVAAPRWVLSGYLALKHPWPGLAEGSGGGGSGRSAGGPLGLWAGGSQVQLVQSGAEVKKPGASVKVSCKASGYTFTTAGMQWVRQAPGQGLEWMGWINTHSGVPKYAEDFKGRVTISADTSTSTAYLQLSSLKSEDTAVYYCARSGFGSSYWYFDVWGQGTLVTVSSASTKGPSVFPLAPSSKSTSGGTAALGCLVKDYFPEPVTVSWNSGALTSGVHTFPAVLQSSGLYSLSSVVTVPSSSLGTQTYICNVNHKPSNTKVDKRVEPKSCDKTHTCPPCPAPELLGGPSVFLFPPKPKDTLMISRTPEVTCVVVDVSHEDPEVKFNWYVDGVEVHNAKTKPREEQYNSTYRVVSVLTVLHQDWLNGKEYKCKVSNKALPAPIEKTISKAKGQPREPQVYTLPPSREEMTKNQVSLTCLVKGFYPSDIAVEWESNGQPENNYKTTPPVLDSDGSFFLYSKLTVDKSRWQQGNVFSCSVMHEALHNHYTQKSLSLSPGK

SEQ ID NO: 16 - protein, 516 aa, synthetic construct
  REGION 1..516: note = Amino acid sequence of the full length of MHT3423 H chain
MKHLWFFLLLVAAPRWVLSGYLALKHPWPGLAEGSGGGGSGRSAGGGGGSGGGGSGGGGSGGGGSQVQLVQSGAEVKKPGASVKVSCKASGYTFTTAGMQWVRQAPGQGLEWMGWINTHSGVPKYAEDFKGRVTISADTSTSTAYLQLSSLKSEDTAVYYCARSGFGSSYWYFDVWGQGTLVTVSSASTKGPSVFPLAPSSKSTSGGTAALGCLVKDYFPEPVTVSWNSGALTSGVHTFPAVLQSSGLYSLSSVVTVPSSSLGTQTYICNVNHKPSNTKVDKRVEPKSCDKTHTCPPCPAPELLGGPSVFLFPPKPKDTLMISRTPEVTCVVVDVSHEDPEVKFNWYVDGVEVHNAKTKPREEQYNSTYRVVSVLTVLHQDWLNGKEYKCKVSNKALPAPIEKTISKAKGQPREPQVYTLPPSREEMTKNQVSLTCLVKGFYPSDIAVEWESNGQPENNYKTTPPVLDSDGSFFLYSKLTVDKSRWQQGNVFSCSVMHEALHNHYTQKSLSLSPGK

SEQ ID NO: 17 - protein, 508 aa, synthetic construct
  REGION 1..508: note = Amino acid sequence of the full length of MHT3203 H chain
MKHLWFFLLLVAAPRWVLSGYLALKHPWPGLAEGSGGGGSGRSANAGGPLFAAPGGSQVQLVQSGAEVKKPGASVKVSCKASGYTFTTAGMQWVRQAPGQGLEWMGWINTHSGVPKYAEDFKGRVTISADTSTSTAYLQLSSLKSEDTAVYYCARSGFGSSYWYFDVWGQGTLVTVSSASTKGPSVFPLAPSSKSTSGGTAALGCLVKDYFPEPVTVSWNSGALTSGVHTFPAVLQSSGLYSLSSVVTVPSSSLGTQTYICNVNHKPSNTKVDKRVEPKSCDKTHTCPPCPAPELLGGPSVFLFPPKPKDTLMISRTPEVTCVVVDVSHEDPEVKFNWYVDGVEVHNAKTKPREEQYNSTYRVVSVLTVLHQDWLNGKEYKCKVSNKALPAPIEKTISKAKGQPREPQVYTLPPSREEMTKNQVSLTCLVKGFYPSDIAVEWESNGQPENNYKTTPPVLDSDGSFFLYSKLTVDKSRWQQGNVFSCSVMHEALHNHYTQKSLSLSPGK

SEQ ID NO: 18 - protein, 465 aa, synthetic construct
  REGION 1..465: note = Amino acid sequence of the full length of hM23H1L1 H chain
MKHLWFFLLLVAAPRWVLSQVQLVQSGAEVKKPGASVKVSCKASGYAFSNYLIEWVRQAPGQGLEWMGVINPGSGVTNYNEKFKGRVTITADTSTSTAYMELSSLRSEDTAVYYCARAEAWFAYWGQGTLVTVSSASTKGPSVFPLAPSSKSTSGGTAALGCLVKDYFPEPVTVSWNSGALTSGVHTFPAVLQSSGLYSLSSVVTVPSSSLGTQTYICNVNHKPSNTKVDKRVEPKSCDKTHTCPPCPAPELLGGPSVFLFPPKPKDTLMISRTPEVTCVVVDVSHEDPEVKFNWYVDGVEVHNAKTKPREEQYNSTYRVVSVLTVLHQDWLNGKEYKCKVSNKALPAPIEKTISKAKGQPREPQVYTLPPSREEMTKNQVSLTCLVKGFYPSDIAVEWESNGQPENNYKTTPPVLDSDGSFFLYSKLTVDKSRWQQGNVFSCSVMHEALHNHYTQKSLSLSPGK

SEQ ID NO: 19 - protein, 240 aa, synthetic construct
  REGION 1..240: note = Amino acid sequence of the full length of hM23H1L1 L chain
MVLQTQVFISLLLWISGAYGDIVMTQSPDSLAVSLGERATINCKSSQSLLYSSNQKNYLAWYQQKPGQPPKLLIYWASTRESGVPDRFSGSGSGTDFTLTISSLQAEDVAVYYCQRYYGYPWTFGQGTKVEIKRTVAAPSVFIFPPSDEQLKSGTASVVCLLNNFYPREAKVQWKVDNALQSGNSQESVTEQDSKDSTYSLSSTLTLSKADYEKHKVYACEVTHQGLSSPVTKSFNRGEC

SEQ ID NO: 20 - protein, 276 aa, synthetic construct
  REGION 1..276: note = Amino acid sequence of the full length of MhM1008 L chain
MVLQTQVFISLLLWISGAYGGENMWNDLDLVPLGILGSGGGGSVLVPMAMMASGGSDIVMTQSPDSLAVSLGERATINCKSSQSLLYSSNQKNYLAWYQQKPGQPPKLLIYWASTRESGVPDRFSGSGSGTDFTLTISSLQAEDVAVYYCQRYYGYPWTFGQGTKVEIKRTVAAPSVFIFPPSDEQLKSGTASVVCLLNNFYPREAKVQWKVDNALQSGNSQESVTEQDSKDSTYSLSSTLTLSKADYEKHKVYACEVTHQGLSSPVTKSFNRGEC

SEQ ID NO: 21 - protein, 276 aa, synthetic construct
  REGION 1..276: note = Amino acid sequence of the full length of MhM1013 L chain
MVLQTQVFISLLLWISGAYGGNFYHQYPWPLEILGSGSGGGGSVLVPMAMMASGGSDIVMTQSPDSLAVSLGERATINCKSSQSLLYSSNQKNYLAWYQQKPGQPPKLLIYWASTRESGVPDRFSGSGSGTDFTLTISSLQAEDVAVYYCQRYYGYPWTFGQGTKVEIKRTVAAPSVFIFPPSDEQLKSGTASVVCLLNNFYPREAKVQWKVDNALQSGNSQESVTEQDSKDSTYSLSSTLTLSKADYEKHKVYACEVTHQGLSSPVTKSFNRGEC

SEQ ID NO: 22 - protein, 465 aa, synthetic construct
  REGION 1..465: note = Amino acid sequence of the full length of hM23-M1 H chain
MKHLWFFLLLVAAPRWVLSQVQLVQSGAEVKKPGASVKVSCKASGAAFSNYLIEWVRQAPGQGLEWMGVINPGSGVTNYNEKFKGRVTITADTSTSTAYMELSSLRSEDTAVYYCARAEAWFAYWGQGTLVTVSSASTKGPSVFPLAPSSKSTSGGTAALGCLVKDYFPEPVTVSWNSGALTSGVHTFPAVLQSSGLYSLSSVVTVPSSSLGTQTYICNVNHKPSNTKVDKRVEPKSCDKTHTCPPCPAPELLGGPSVFLFPPKPKDTLMISRTPEVTCVVVDVSHEDPEVKFNWYVDGVEVHNAKTKPREEQYNSTYRVVSVLTVLHQDWLNGKEYKCKVSNKALPAPIEKTISKAKGQPREPQVYTLPPSREEMTKNQVSLTCLVKGFYPSDIAVEWESNGQPENNYKTTPPVLDSDGSFFLYSKLTVDKSRWQQGNVFSCSVMHEALHNHYTQKSLSLSPGK

SEQ ID NO: 23 - protein, 240 aa, synthetic construct
  REGION 1..240: note = Amino acid sequence of the full length of hM23-M1 L chain
MVLQTQVFISLLLWISGAYGDIVMTQSPDSLAVSLGERATINCKSSQSLLYSSNQKNYLAWYQQKPGQPPKLLIYWASTRESGVPDRFSGSGSGTDFTLTISSLQAEDVAVYYCQRYYGYPWTFGQGTKVEIKRAVAAPSVFIFPPSDEQLKSGTASVVCLLNNFYPREAKVQWKVDNALQSGNSQESVTEQDSKDSTYSLSSTLTLSKADYEKHKVYACEVTHQGLSSPVTKSFNRGEC

SEQ ID NO: 24 - protein, 276 aa, synthetic construct
  REGION 1..276: note = Amino acid sequence of the full length of MhM1018-M1 L chain
MVLQTQVFISLLLWISGAYGGNFYHQYPWPLEILGSGSGGGGSGGGGSGGGGSGGSDIVMTQSPDSLAVSLGERATINCKSSQSLLYSSNQKNYLAWYQQKPGQPPKLLIYWASTRESGVPDRFSGSGSGTDFTLTISSLQAEDVAVYYCQRYYGYPWTFGQGTKVEIKRTVAAPSVFIFPPSDEQLKSGTASVVCLLNNFYPREAKVQWKVDNALQSGNSQESVTEQDSKDSTYSLSSTLTLSKADYEKHKVYACEVTHQGLSSPVTKSFNRGEC

SEQ ID NO: 25 - protein, 278 aa, synthetic construct
  REGION 1..278: note = Amino acid sequence of the full length of MhM1019-M1 L chain
MVLQTQVFISLLLWISGAYGGNFYHQYPWPLEILGSGGGGSGRSANAGGSGGGGSGGSDIVMTQSPDSLAVSLGERATINCKSSQSLLYSSNQKNYLAWYQQKPGQPPKLLIYWASTRESGVPDRFSGSGSGTDFTLTISSLQAEDVAVYYCQRYYGYPWTFGQGTKVEIKRTVAAPSVFIFPPSDEQLKSGTASVVCLLNNFYPREAKVQWKVDNALQSGNSQESVTEQDSKDSTYSLSSTLTLSKADYEKHKVYACEVTHQGLSSPVTKSFNRGEC

SEQ ID NO: 26 - protein, 278 aa, synthetic construct
  REGION 1..278: note = Amino acid sequence of the full length of MhM1020-M1 L chain
MVLQTQVFISLLLWISGAYGGNFYHQYPWPLEILGSGGGGSGGGGSGGGPLFAAPGGSDIVMTQSPDSLAVSLGERATINCKSSQSLLYSSNQKNYLAWYQQKPGQPPKLLIYWASTRESGVPDRFSGSGSGTDFTLTISSLQAEDVAVYYCQRYYGYPWTFGQGTKVEIKRTVAAPSVFIFPPSDEQLKSGTASVVCLLNNFYPREAKVQWKVDNALQSGNSQESVTEQDSKDSTYSLSSTLTLSKADYEKHKVYACEVTHQGLSSPVTKSFNRGEC

SEQ ID NO: 27 - protein, 278 aa, synthetic construct
  REGION 1..278: note = Amino acid sequence of the full length of MhM1021-M1 L chain
MVLQTQVFISLLLWISGAYGGNFYHQYPWPLEILGSGGGGSGRSANAGGPLFAAPGGSDIVMTQSPDSLAVSLGERATINCKSSQSLLYSSNQKNYLAWYQQKPGQPPKLLIYWASTRESGVPDRFSGSGSGTDFTLTISSLQAEDVAVYYCQRYYGYPWTFGQGTKVEIKRTVAAPSVFIFPPSDEQLKSGTASVVCLLNNFYPREAKVQWKVDNALQSGNSQESVTEQDSKDSTYSLSSTLTLSKADYEKHKVYACEVTHQGLSSPVTKSFNRGEC

SEQ ID NO: 28 - protein, 278 aa, synthetic construct
  REGION 1..278: note = Amino acid sequence of the full length of MhM1022-M1 L chain
MVLQTQVFISLLLWISGAYGGNFYHQYPWPLEILGSGGGGSPLGLAGGGSGGGGSGGSDIVMTQSPDSLAVSLGERATINCKSSQSLLYSSNQKNYLAWYQQKPGQPPKLLIYWASTRESGVPDRFSGSGSGTDFTLTISSLQAEDVAVYYCQRYYGYPWTFGQGTKVEIKRTVAAPSVFIFPPSDEQLKSGTASVVCLLNNFYPREAKVQWKVDNALQSGNSQESVTEQDSKDSTYSLSSTLTLSKADYEKHKVYACEVTHQGLSSPVTKSFNRGEC

SEQ ID NO: 29 - protein, 278 aa, synthetic construct
  REGION 1..278: note = Amino acid sequence of the full length of MhM1023-M1 L chain
MVLQTQVFISLLLWISGAYGGNFYHQYPWPLEILGSGGGGSPLGLAGGGPLFAAPGGSDIVMTQSPDSLAVSLGERATINCKSSQSLLYSSNQKNYLAWYQQKPGQPPKLLIYWASTRESGVPDRFSGSGSGTDFTLTISSLQAEDVAVYYCQRYYGYPWTFGQGTKVEIKRTVAAPSVFIFPPSDEQLKSGTASVVCLLNNFYPREAKVQWKVDNALQSGNSQESVTEQDSKDSTYSLSSTLTLSKADYEKHKVYACEVTHQGLSSPVTKSFNRGEC

SEQ ID NO: 30 - protein, 468 aa, synthetic construct
  REGION 1..468: note = Amino acid sequence of the full length of Cetuximab H chain
MKHLWFFLLLVAAPRWVLSQVQLKQSGPGLVQPSQSLSITCTVSGFSLTNYGVHWVRQSPGKGLEWLGVIWSGGNTDYNTPFTSRLSINKDNSKSQVFFKMNSLQSNDTAIYYCARALTYYDYEFAYWGQGTLVTVSAASTKGPSVFPLAPSSKSTSGGTAALGCLVKDYFPEPVTVSWNSGALTSGVHTFPAVLQSSGLYSLSSVVTVPSSSLGTQTYICNVNHKPSNTKVDKRVEPKSCDKTHTCPPCPAPELLGGPSVFLFPPKPKDTLMISRTPEVTCVVVDVSHEDPEVKFNWYVDGVEVHNAKTKPREEQYNSTYRVVSVLTVLHQDWLNGKEYKCKVSNKALPAPIEKTISKAKGQPREPQVYTLPPSREEMTKNQVSLTCLVKGFYPSDIAVEWESNGQPENNYKTTPPVLDSDGSFFLYSKLTVDKSRWQQGNVFSCSVMHEALHNHYTQKSLSLSPGK

SEQ ID NO: 31 - protein, 234 aa, synthetic construct
  REGION 1..234: note = Amino acid sequence of the full length of Cetuximab L chain
MVLQTQVFISLLLWISGAYGDILLTQSPVILSVSPGERVSFSCRASQSIGTNIHWYQQRTNGSPRLLIKYASESISGIPSRFSGSGSGTDFTLSINSVESEDIADYYCQQNNNWPTTFGAGTKLELKRTVAAPSVFIFPPSDEQLKSGTASVVCLLNNFYPREAKVQWKVDNALQSGNSQESVTEQDSKDSTYSLSSTLTLSKADYEKHKVYACEVTHQGLSSPVTKSFNRGEC

SEQ ID NO: 32 - protein, 464 aa, synthetic construct
  REGION 1..464: note = Amino acid sequence of the full length of C3022 H chain
MKHLWFFLLLVAAPRWVLSQVQLVQSGAEVKKPGASVKVSCKASGYTFTGYYMHWVRQAPGQGLEWMGRINPNSGGTNYAQKFQGRVTMTRDTSISTAYMELSGLRSDDTAVYYCASGSVRHPWGQGTLVTVSSASTKGPSVFPLAPSSKSTSGGTAALGCLVKDYFPEPVTVSWNSGALTSGVHTFPAVLQSSGLYSLSSVVTVPSSSLGTQTYICNVNHKPSNTKVDKRVEPKSCDKTHTCPPCPAPELLGGPSVFLFPPKPKDTLMISRTPEVTCVVVDVSHEDPEVKFNWYVDGVEVHNAKTKPREEQYNSTYRVVSVLTVLHQDWLNGKEYKCKVSNKALPAPIEKTISKAKGQPREPQVYTLPPSREEMTKNQVSLTCLVKGFYPSDIAVEWESNGQPENNYKTTPPVLDSDGSFFLYSKLTVDKSRWQQGNVFSCSVMHEALHNHYTQKSLSLSPGK

SEQ ID NO: 33 - protein, 236 aa, synthetic construct
  REGION 1..236: note = Amino acid sequence of the full length of C3022 L chain
MVLQTQVFISLLLWISGAYGQPVLTQPPSASGTPGQRVTISCSGSRSNIGGNIVSWYQQFPGTAPRLLTYADNQRPSGVPDRFSGSKSGTSASLAISGLQSEDEADYYCAAWDDSLNGVVFGGGTKLTVLGQPKAAPSVTLFPPSSEELQANKATLVCLISDFYPGAVTVAWKADSSPVKAGVETTTPSKQSNNKYAASSYLSLTPEQWKSHRSYSCQVTHEGSTVEKTVAPTECS

SEQ ID NO: 34 - protein, 273 aa, synthetic construct
  REGION 1..273: note = Amino acid sequence of the full length of MCE-2105 L chain
MVLQTQVFISLLLWISGAYGMGLMHMEKSRSWYLSRQGGGGSGRSANAGGPLFAAPGGSDILLTQSPVILSVSPGERVSFSCRASQSIGTNIHWYQQRTNGSPRLLIKYASESISGIPSRFSGSGSGTDFTLSINSVESEDIADYYCQQNNNWPTTFGAGTKLELKRTVAAPSVFIFPPSDEQLKSGTASVVCLLNNFYPREAKVQWKVDNALQSGNSQESVTEQDSKDSTYSLSSTLTLSKADYEKHKVYACEVTHQGLSSPVTKSFNRGEC

SEQ ID NO: 35 - protein, 502 aa, synthetic construct
  REGION 1..502: note = Amino acid sequence of the full length of MC3-9003 H chain
MKHLWFFLLLVAAPRWVLSGETMSVFTRDYFTETPGGGGSGRSANAGGPLFAAPGGSQVQLVQSGAEVKKPGASVKVSCKASGYTFTGYYMHWVRQAPGQGLEWMGRINPNSGGTNYAQKFQGRVTMTRDTSISTAYMELSGLRSDDTAVYYCASGSVRHPWGQGTLVTVSSASTKGPSVFPLAPSSKSTSGGTAALGCLVKDYFPEPVTVSWNSGALTSGVHTFPAVLQSSGLYSLSSVVTVPSSSLGTQTYICNVNHKPSNTKVDKRVEPKSCDKTHTCPPCPAPELLGGPSVFLFPPKPKDTLMISRTPEVTCVVVDVSHEDPEVKFNWYVDGVEVHNAKTKPREEQYNSTYRVVSVLTVLHQDWLNGKEYKCKVSNKALPAPIEKTISKAKGQPREPQVYTLPPSREEMTKNQVSLTCLVKGFYPSDIAVEWESNGQPENNYKTTPPVLDSDGSFFLYSKLTVDKSRWQQGNVFSCSVMHEALHNHYTQKSLSLSPGK

SEQ ID NO: 36 - protein, 10 aa, synthetic construct
  REGION 1..9: note = Synthetic
SGRSANAILE

SEQ ID NO: 37 - protein, 7 aa, synthetic construct
  REGION 1..7: note = Synthetic
SGRSANA

SEQ ID NO: 38 - protein, 5 aa, synthetic construct
  REGION 1..5: note = Synthetic
SGRSA

SEQ ID NO: 39 - protein, 10 aa, synthetic construct
  REGION 1..10: note = Synthetic
VLVPMAMMAS

SEQ ID NO: 40 - protein, 6 aa, synthetic construct
  REGION 1..6: note = Synthetic
PLGLWA

SEQ ID NO: 41 - protein, 6 aa, synthetic construct
  REGION 1..6: note = Synthetic
PLGLAG

SEQ ID NO: 42 - protein, 508 aa, synthetic construct
  REGION 1..508: note = Amino acid sequence of the full length of MHT1903 H chain
MKHLWFFLLLVAAPRWVLSGYLALKHPWPGLAEGSGGGGSGRSANAGGSGGGGSGGSQVQLVQSGAEVKKPGASVKVSCKASGYTFTTAGMQWVRQAPGQGLEWMGWINTHSGVPKYAEDFKGRVTISADTSTSTAYLQLSSLKSEDTAVYYCARSGFGSSYWYFDVWGQGTLVTVSSASTKGPSVFPLAPSSKSTSGGTAALGCLVKDYFPEPVTVSWNSGALTSGVHTFPAVLQSSGLYSLSSVVTVPSSSLGTQTYICNVNHKPSNTKVDKRVEPKSCDKTHTCPPCPAPELLGGPSVFLFPPKPKDTLMISRTPEVTCVVVDVSHEDPEVKFNWYVDGVEVHNAKTKPREEQYNSTYRVVSVLTVLHQDWLNGKEYKCKVSNKALPAPIEKTISKAKGQPREPQVYTLPPSREEMTKNQVSLTCLVKGFYPSDIAVEWESNGQPENNYKTTPPVLDSDGSFFLYSKLTVDKSRWQQGNVFSCSVMHEALHNHYTQKSLSLSPGK

SEQ ID NO: 43 - protein, 508 aa, synthetic construct
  REGION 1..508: note = Amino acid sequence of the full length of MHT3219 H chain
MKHLWFFLLLVAAPRWVLSGYLALKHPWPGLAEGSGGGGPLFAAPGGSGRSANAGGSQVQLVQSGAEVKKPGASVKVSCKASGYTFTTAGMQWVRQAPGQGLEWMGWINTHSGVPKYAEDFKGRVTISADTSTSTAYLQLSSLKSEDTAVYYCARSGFGSSYWYFDVWGQGTLVTVSSASTKGPSVFPLAPSSKSTSGGTAALGCLVKDYFPEPVTVSWNSGALTSGVHTFPAVLQSSGLYSLSSVVTVPSSSLGTQTYICNVNHKPSNTKVDKRVEPKSCDKTHTCPPCPAPELLGGPSVFLFPPKPKDTLMISRTPEVTCVVVDVSHEDPEVKFNWYVDGVEVHNAKTKPREEQYNSTYRVVSVLTVLHQDWLNGKEYKCKVSNKALPAPIEKTISKAKGQPREPQVYTLPPSREEMTKNQVSLTCLVKGFYPSDIAVEWESNGQPENNYKTTPPVLDSDGSFFLYSKLTVDKSRWQQGNVFSCSVMHEALHNHYTQKSLSLSPGK

SEQ ID NO: 44 - protein, 6 aa, synthetic construct
  REGION 1..6: note = Amino acid sequence of CAPN substrate
FVFAMR

SEQ ID NO: 45 - protein, 6 aa, synthetic construct
  REGION 1..6: note = Amino acid sequence of CAPN substrate
FLFMVR

SEQ ID NO: 46 - protein, 6 aa, synthetic construct
  REGION 1..6: note = Amino acid sequence of CAPN substrate
FLFTMW

SEQ ID NO: 47 - protein, 6 aa, synthetic construct
  REGION 1..6: note = Amino acid sequence of CAPN substrate
LVFAVP

SEQ ID NO: 48 - protein, 6 aa, synthetic construct
  REGION 1..6: note = Amino acid sequence of CAPN substrate
FVFAWR

SEQ ID NO: 49 - protein, 6 aa, synthetic construct
  REGION 1..6: note = Amino acid sequence of CAPN substrate
FLFARM

SEQ ID NO: 50 - protein, 6 aa, synthetic construct
  REGION 1..6: note = Amino acid sequence of CAPN substrate
LLFSGR

SEQ ID NO: 51 - protein, 6 aa, synthetic construct
  REGION 1..6: note = Amino acid sequence of CAPN substrate
LLFGMR

SEQ ID NO: 52 - protein, 6 aa, synthetic construct
  REGION 1..6: note = Amino acid sequence of CAPN substrate
LFALRW

SEQ ID NO: 53 - protein, 6 aa, synthetic construct
  REGION 1..6: note = Amino acid sequence of CAPN substrate
LLFASW

SEQ ID NO: 54 - protein, 508 aa, synthetic construct
  REGION 1..508: note = Amino acid sequence of the full length of MHT5082 H chain
MKHLWFFLLLVAAPRWVLSGYLALKHPWPGLAEGSGGGGSGRSANAGGFVFAMRGGSQVQLVQSGAEVKKPGASVKVSCKASGYTFTTAGMQWVRQAPGQGLEWMGWINTHSGVPKYAEDFKGRVTISADTSTSTAYLQLSSLKSEDTAVYYCARSGFGSSYWYFDVWGQGTLVTVSSASTKGPSVFPLAPSSKSTSGGTAALGCLVKDYFPEPVTVSWNSGALTSGVHTFPAVLQSSGLYSLSSVVTVPSSSLGTQTYICNVNHKPSNTKVDKRVEPKSCDKTHTCPPCPAPELLGGPSVFLFPPKPKDTLMISRTPEVTCVVVDVSHEDPEVKFNWYVDGVEVHNAKTKPREEQYNSTYRVVSVLTVLHQDWLNGKEYKCKVSNKALPAPIEKTISKAKGQPREPQVYTLPPSREEMTKNQVSLTCLVKGFYPSDIAVEWESNGQPENNYKTTPPVLDSDGSFFLYSKLTVDKSRWQQGNVFSCSVMHEALHNHYTQKSLSLSPGK

SEQ ID NO: 55 - protein, 508 aa, synthetic construct
  REGION 1..508: note = Amino acid sequence of the full length of MHT5084 H chain
MKHLWFFLLLVAAPRWVLSGYLALKHPWPGLAEGSGGGGSGRSANAGGFLFMVRGGSQVQLVQSGAEVKKPGASVKVSCKASGYTFTTAGMQWVRQAPGQGLEWMGWINTHSGVPKYAEDFKGRVTISADTSTSTAYLQLSSLKSEDTAVYYCARSGFGSSYWYFDVWGQGTLVTVSSASTKGPSVFPLAPSSKSTSGGTAALGCLVKDYFPEPVTVSWNSGALTSGVHTFPAVLQSSGLYSLSSVVTVPSSSLGTQTYICNVNHKPSNTKVDKRVEPKSCDKTHTCPPCPAPELLGGPSVFLFPPKPKDTLMISRTPEVTCVVVDVSHEDPEVKFNWYVDGVEVHNAKTKPREEQYNSTYRVVSVLTVLHQDWLNGKEYKCKVSNKALPAPIEKTISKAKGQPREPQVYTLPPSREEMTKNQVSLTCLVKGFYPSDIAVEWESNGQPENNYKTTPPVLDSDGSFFLYSKLTVDKSRWQQGNVFSCSVMHEALHNHYTQKSLSLSPGK

SEQ ID NO: 56 - protein, 508 aa, synthetic construct
  REGION 1..508: note = Amino acid sequence of the full length of MHT5085 H chain
MKHLWFFLLLVAAPRWVLSGYLALKHPWPGLAEGSGGGGSGRSANAGGFLFTMWGGSQVQLVQSGAEVKKPGASVKVSCKASGYTFTTAGMQWVRQAPGQGLEWMGWINTHSGVPKYAEDFKGRVTISADTSTSTAYLQLSSLKSEDTAVYYCARSGFGSSYWYFDVWGQGTLVTVSSASTKGPSVFPLAPSSKSTSGGTAALGCLVKDYFPEPVTVSWNSGALTSGVHTFPAVLQSSGLYSLSSVVTVPSSSLGTQTYICNVNHKPSNTKVDKRVEPKSCDKTHTCPPCPAPELLGGPSVFLFPPKPKDTLMISRTPEVTCVVVDVSHEDPEVKFNWYVDGVEVHNAKTKPREEQYNSTYRVVSVLTVLHQDWLNGKEYKCKVSNKALPAPIEKTISKAKGQPREPQVYTLPPSREEMTKNQVSLTCLVKGFYPSDIAVEWESNGQPENNYKTTPPVLDSDGSFFLYSKLTVDKSRWQQGNVFSCSVMHEALHNHYTQKSLSLSPGK

SEQ ID NO: 57 - protein, 508 aa, synthetic construct
  REGION 1..508: note = Amino acid sequence of the full length of MHT5086 H chain
MKHLWFFLLLVAAPRWVLSGYLALKHPWPGLAEGSGGGGSGRSANAGGLVFAVPGGSQVQLVQSGAEVKKPGASVKVSCKASGYTFTTAGMQWVRQAPGQGLEWMGWINTHSGVPKYAEDFKGRVTISADTSTSTAYLQLSSLKSEDTAVYYCARSGFGSSYWYFDVWGQGTLVTVSSASTKGPSVFPLAPSSKSTSGGTAALGCLVKDYFPEPVTVSWNSGALTSGVHTFPAVLQSSGLYSLSSVVTVPSSSLGTQTYICNVNHKPSNTKVDKRVEPKSCDKTHTCPPCPAPELLGGPSVFLFPPKPKDTLMISRTPEVTCVVVDVSHEDPEVKFNWYVDGVEVHNAKTKPREEQYNSTYRVVSVLTVLHQDWLNGKEYKCKVSNKALPAPIEKTISKAKGQPREPQVYTLPPSREEMTKNQVSLTCLVKGFYPSDIAVEWESNGQPENNYKTTPPVLDSDGSFFLYSKLTVDKSRWQQGNVFSCSVMHEALHNHYTQKSLSLSPGK

SEQ ID NO: 58 - protein, 508 aa, synthetic construct
  REGION 1..508: note = Amino acid sequence of the full length of MHT5090 H chain
MKHLWFFLLLVAAPRWVLSGYLALKHPWPGLAEGSGGGGSGRSANAGGFVFAWRGGSQVQLVQSGAEVKKPGASVKVSCKASGYTFTTAGMQWVRQAPGQGLEWMGWINTHSGVPKYAEDFKGRVTISADTSTSTAYLQLSSLKSEDTAVYYCARSGFGSSYWYFDVWGQGTLVTVSSASTKGPSVFPLAPSSKSTSGGTAALGCLVKDYFPEPVTVSWNSGALTSGVHTFPAVLQSSGLYSLSSVVTVPSSSLGTQTYICNVNHKPSNTKVDKRVEPKSCDKTHTCPPCPAPELLGGPSVFLFPPKPKDTLMISRTPEVTCVVVDVSHEDPEVKFNWYVDGVEVHNAKTKPREEQYNSTYRVVSVLTVLHQDWLNGKEYKCKVSNKALPAPIEKTISKAKGQPREPQVYTLPPSREEMTKNQVSLTCLVKGFYPSDIAVEWESNGQPENNYKTTPPVLDSDGSFFLYSKLTVDKSRWQQGNVFSCSVMHEALHNHYTQKSLSLSPGK

SEQ ID NO: 59 - protein, 508 aa, synthetic construct
  REGION 1..508: note = Amino acid sequence of the full length of MHT5091 H chain
MKHLWFFLLLVAAPRWVLSGYLALKHPWPGLAEGSGGGGSGRSANAGGFLFARMGGSQVQLVQSGAEVKKPGASVKVSCKASGYTFTTAGMQWVRQAPGQGLEWMGWINTHSGVPKYAEDFKGRVTISADTSTSTAYLQLSSLKSEDTAVYYCARSGFGSSYWYFDVWGQGTLVTVSSASTKGPSVFPLAPSSKSTSGGTAALGCLVKDYFPEPVTVSWNSGALTSGVHTFPAVLQSSGLYSLSSVVTVPSSSLGTQTYICNVNHKPSNTKVDKRVEPKSCDKTHTCPPCPAPELLGGPSVFLFPPKPKDTLMISRTPEVTCVVVDVSHEDPEVKFNWYVDGVEVHNAKTKPREEQYNSTYRVVSVLTVLHQDWLNGKEYKCKVSNKALPAPIEKTISKAKGQPREPQVYTLPPSREEMTKNQVSLTCLVKGFYPSDIAVEWESNGQPENNYKTTPPVLDSDGSFFLYSKLTVDKSRWQQGNVFSCSVMHEALHNHYTQKSLSLSPGK

SEQ ID NO: 60 - protein, 508 aa, synthetic construct
  REGION 1..508: note = Amino acid sequence of the full length of MHT5092 H chain
MKHLWFFLLLVAAPRWVLSGYLALKHPWPGLAEGSGGGGSGRSANAGGLLFSGRGGSQVQLVQSGAEVKKPGASVKVSCKASGYTFTTAGMQWVRQAPGQGLEWMGWINTHSGVPKYAEDFKGRVTISADTSTSTAYLQLSSLKSEDTAVYYCARSGFGSSYWYFDVWGQGTLVTVSSASTKGPSVFPLAPSSKSTSGGTAALGCLVKDYFPEPVTVSWNSGALTSGVHTFPAVLQSSGLYSLSSVVTVPSSSLGTQTYICNVNHKPSNTKVDKRVEPKSCDKTHTCPPCPAPELLGGPSVFLFPPKPKDTLMISRTPEVTCVVVDVSHEDPEVKFNWYVDGVEVHNAKTKPREEQYNSTYRVVSVLTVLHQDWLNGKEYKCKVSNKALPAPIEKTISKAKGQPREPQVYTLPPSREEMTKNQVSLTCLVKGFYPSDIAVEWESNGQPENNYKTTPPVLDSDGSFFLYSKLTVDKSRWQQGNVFSCSVMHEALHNHYTQKSLSLSPGK

SEQ ID NO: 61 - protein, 508 aa, synthetic construct
  REGION 1..508: note = Amino acid sequence of the full length of MHT5093 H chain
MKHLWFFLLLVAAPRWVLSGYLALKHPWPGLAEGSGGGGSGRSANAGGLLFGMRGGSQVQLVQSGAEVKKPGASVKVSCKASGYTFTTAGMQWVRQAPGQGLEWMGWINTHSGVPKYAEDFKGRVTISADTSTSTAYLQLSSLKSEDTAVYYCARSGFGSSYWYFDVWGQGTLVTVSSASTKGPSVFPLAPSSKSTSGGTAALGCLVKDYFPEPVTVSWNSGALTSGVHTFPAVLQSSGLYSLSSVVTVPSSSLGTQTYICNVNHKPSNTKVDKRVEPKSCDKTHTCPPCPAPELLGGPSVFLFPPKPKDTLMISRTPEVTCVVVDVSHEDPEVKFNWYVDGVEVHNAKTKPREEQYNSTYRVVSVLTVLHQDWLNGKEYKCKVSNKALPAPIEKTISKAKGQPREPQVYTLPPSREEMTKNQVSLTCLVKGFYPSDIAVEWESNGQPENNYKTTPPVLDSDGSFFLYSKLTVDKSRWQQGNVFSCSVMHEALHNHYTQKSLSLSPGK

SEQ ID NO: 62 - protein, 508 aa, synthetic construct
  REGION 1..508: note = Amino acid sequence of the full length of MHT5094 H chain
MKHLWFFLLLVAAPRWVLSGYLALKHPWPGLAEGSGGGGSGRSANAGGLFALRWGGSQVQLVQSGAEVKKPGASVKVSCKASGYTFTTAGMQWVRQAPGQGLEWMGWINTHSGVPKYAEDFKGRVTISADTSTSTAYLQLSSLKSEDTAVYYCARSGFGSSYWYFDVWGQGTLVTVSSASTKGPSVFPLAPSSKSTSGGTAALGCLVKDYFPEPVTVSWNSGALTSGVHTFPAVLQSSGLYSLSSVVTVPSSSLGTQTYICNVNHKPSNTKVDKRVEPKSCDKTHTCPPCPAPELLGGPSVFLFPPKPKDTLMISRTPEVTCVVVDVSHEDPEVKFNWYVDGVEVHNAKTKPREEQYNSTYRVVSVLTVLHQDWLNGKEYKCKVSNKALPAPIEKTISKAKGQPREPQVYTLPPSREEMTKNQVSLTCLVKGFYPSDIAVEWESNGQPENNYKTTPPVLDSDGSFFLYSKLTVDKSRWQQGNVFSCSVMHEALHNHYTQKSLSLSPGK

SEQ ID NO: 63 - protein, 508 aa, synthetic construct
  REGION 1..508: note = Amino acid sequence of the full length of MHT5095 H chain
MKHLWFFLLLVAAPRWVLSGYLALKHPWPGLAEGSGGGGSGRSANAGGLLFASWGGSQVQLVQSGAEVKKPGASVKVSCKASGYTFTTAGMQWVRQAPGQGLEWMGWINTHSGVPKYAEDFKGRVTISADTSTSTAYLQLSSLKSEDTAVYYCARSGFGSSYWYFDVWGQGTLVTVSSASTKGPSVFPLAPSSKSTSGGTAALGCLVKDYFPEPVTVSWNSGALTSGVHTFPAVLQSSGLYSLSSVVTVPSSSLGTQTYICNVNHKPSNTKVDKRVEPKSCDKTHTCPPCPAPELLGGPSVFLFPPKPKDTLMISRTPEVTCVVVDVSHEDPEVKFNWYVDGVEVHNAKTKPREEQYNSTYRVVSVLTVLHQDWLNGKEYKCKVSNKALPAPIEKTISKAKGQPREPQVYTLPPSREEMTKNQVSLTCLVKGFYPSDIAVEWESNGQPENNYKTTPPVLDSDGSFFLYSKLTVDKSRWQQGNVFSCSVMHEALHNHYTQKSLSLSPGK

SEQ ID NO: 64 - protein, 20 aa, synthetic construct
  REGION 1..20: note = Amino acid sequence of an MMP linker
GSGGGGSGGGSPLGLWAGGS